European Patent Application EP 4 321 020 A1, published February 14, 2024. Title: Oral vaccine composition. Applicant: KAICO Ltd. Kagoshima University Kyushu University. The sequence listing filed with the application follows.

SEQUENCE LISTING (1 sequence)

SEQ ID NO: 1 - protein, 233 aa, Porcine circovirus 2
MTYPRRRYRRRRHRPRSHLGQILRRRPWLVHPRHRYRWRRKNGIFNTRLSRTFGYTVKRTTVTTPSWAVDMMRFKIDDFVPPGGGTNKISIPFEYYRIRKVKVEFWPCSPITQGDRGVGSTAVILDDNFVTKATALTYDPYVNYSSRHTIPQPFSYHSRYFTPKPVLDSTIDYFQPNNKRNQLWLRLQTSGNVDHVGLGAAFENSKYDQDYNIRVTMYVQFREFNLKDPPLKP